European Patent Specification EP 4 065 733 B1, published May 1, 2024. Title: Method and system for detection of extraintestinal E. coli strains pathogenic to poultry. Applicant: Proteon Pharmaceuticals S.A. The sequence listing filed with the application follows.

SEQUENCE LISTING (9 sequences)

SEQ ID NO: 1 - DNA, 20 bp, artificial
  primer
actatgtgcgccgtggttat

SEQ ID NO: 2 - DNA, 20 bp, artificial
  primer
gtgaacgggtgtcgatcagt

SEQ ID NO: 3 - DNA, 20 bp, artificial
  primer
gagcacctactccacaagcg

SEQ ID NO: 4 - DNA, 20 bp, artificial
  primer
tcgggcaaccaacaaaggta

SEQ ID NO: 5 - DNA, 25 bp, artificial
  primer
cacaactctcggcaatatatcatca

SEQ ID NO: 6 - DNA, 22 bp, artificial
  primer
tatgggtttggtggtacgtagt

SEQ ID NO: 7 - DNA, 3786 bp, Escherichia coli
atgataatcatatgccagcacccatccaggagtcatgcatccataacaatgcgggaccggagcgtgctggcttttttgcggaacgatccggccagtggatcgtattttacagacggaggaggcttaatgcctgcgaatcacactcccacaccggctcagtcatggatagttcgcctggcgcgcgtgtgctgggaacgtaagaaacttagtgtcatcgtggtggtagcgtcagtatcgactattttgctggctgcgctgacgccactgctgacaagacaggctgtgaatgacgcactggcgggcaatccggcccgcctgccgtggctggcctgcgggttactgttgatcgctttttttgatttcatcggtaactatgtgcgccgtggttatgccgggatgctctcactctgggtgcagcataccctcagaggacgggtattcgacagtattcagaaacttgacggcgcaggccaggatgcgctgcgcaccgggcaggtgatttcacggaccaacagcgatctgcagcaggtgcataccctgctgcagatgtgcccggtgccgctggcagtgttcacttattacattgccggcattgccgtgatgctgtggatgtcccctgccatgacgcttatcgtcgtgtgcgtactggtatgcctggcgatcaccgcgcttcgtgcgcgtcgtagggtcttcgcgcaaaccgggctggcctcggaccaactggcgaatctcaccgaacatatacgcgaggtgctggcacagatctcagtggtaaaatcctgtgtggcagagatgcgtgaaacgcactggctcgataggcagtcgcggcagattgtgcgtgtacgcatcggtgcggttatctcgcaggcgatgcctggggccaccatgctggcgctaccggtgctcgggcaaatcgtcctgctgtgctacggcgggtggtcggtcatgcacgggcggatcgatctcggtaccttcgttgcattcgccagcttcctcgcgatgctgaccgggccaacccgcgtactggcatcgtttctggttatcgcacagcgcactcaggcgtccgtggagcgggtgtttgcactgatcgacacccgttcacagatggaggacgggacggagtcgattaacagtcaggttgtcggactggaactggagaatatgagctttgactaccaccatggcgacagacatatcctcagcaatatctccttttccctgcgcgccggtgaaaccgtggcggtggtgggcgcatcgggttcaggaaaatcgaccctgttgatgctactggcgcgtttttatgatccctgctccggaaagatatggctcaacaccagcgaaggccgacaaaatcttcgcgatatcagactggaggcgcttcgtcgccgggtaggcatcgtatttgaagatgcttttctgtttgccggtacggtggcggaaaatatcgcctatggccaccctcaggcaacggcggacgacattcgccgtgcggcagctgctgcaggagccagcgattttattaacgccctgccgaaaggcttcgatagcctgttaaccgaacggggtacgaatctttccggcgggcagaggcagcgaatagcgctggcgcgggcgctcattactgcaccggacgtgttaatcctggatgatactacctcagcggttgatgctgttacggaagcggagattaataccgcgctgggtcgctatgctgacgaagggcatatgctgctggtgattgcccgacggcgttcaacacttcagctagccagccgggttgtggtgctggataagggccgtatggtggataccggaaccccggcagaacttgaagcgcgctgtccggcgttccgcgcactgatgaccggcgacagcgattttctggccacgtcccacaatagccacaacgaattgtggccggctgaaccagcgacacaagacgatgtaacggatacgggggataaaggttttgtcgcccgtatgacccgcgtaccggaaaatgcagtacagcaggcgctggccggtaaaggtcgcaaagtcacgtcactactgaagcctgtggcgtggatgttcgtcatcgccgctctgctgatcgcactcgattctgcggcaggcgtaggggtactgatactgttgcagcacggcattgactccggtgtcgccgcaggcgatatgtcgatcatcggcctctgtgccctgctcgccctgtgcctggtcattgtgggctggtgcagttattctctgcagacggtcttcgccgccagagcggcggaatcagttcagcattcggtgcgcttgcgcagcttcggccatatgctgcgtcttggactcccctggcatgaaaagcatgccgattcgcgtcttacccgcatgaccgttgatgtggactctctcgcccgctttctgcaaaacggccttgccggtgcggccaccagtctggtgacgatgttcgcaatcgccgccaccatgttctggctcgacccgttcctggcgctgacggcattaagcgcagtgccagtggccgcactggcaaccatgatttatcgccgcctcagtacccctgcttatgcacaggcacggctggaaataggcaaagtcaacagcaccctgcaggaaaaagtctctggcctgcgtgtcgtgcaatcgcatggtcagcaggaactggagggcgcccggctgcgcgcgttatcggagcgtttccgcgcaacccgtgtgcgagcacaaaaataccttgcagtctattttccgttcctgacattctgcaccgaggcctcctatgccgctgttctgttagtgggagcttcgcaggtcgccgctggagaaatgactgccggggtactggcggctttcttcctgttgctggggcaattctatgggccagtgcagcagttatcagggattgtcgacgcctggcagcaggcgacagccagcggcaaacatattgatgaactactggcgacagaaggcactgagaacctcgggtcctcttcggtcctccctgtcaccggtgcactgcatcttgatgaggtcacgttcagttatcccgacagtcacgagccagctctgaacaaacttaccctgacgatccctgagggaatggttgtcgcggtcgtcggtcgcagcggtgcgggtaagtcgacgctgattaagctgattgccgggttgtatttccccacgcacggcaacatcagaatcggtgtgcaaatgctcgatgatgcctcgctcactgagtatcgtcgccagattgggcttgtcgatcaggatgtagcactgtttagtagtgatattgcagaaaacattcgttattcacggccatccgccaccaatgaagacgttgaaattgcctcacagcgggcagggctgtatgagatggtgtgcaatctgccgcagggattccggacaccggtgaataacggcggagccgatctgcccgcaggtcagcgccagttgattgcgctggcccgcgcgcaactggcgaatgcccacatcctgctgctcgacgaagccacgtcatgtctggatcgcacatccgaagaacgactgatgtcatcgttaacagatgtcgtgcatgccgggaagcactcggcgctgattgttgcacatcgtctgaccaccgcgcaacgctgcgatctgattgccgttattgataaggggttacttgcggaatacggaacccacgaacagctgttatctgcgggcggcctctatacccgcttatggcatgacagcgtcagcagtactgctctccatcgccagcacaacatgaaggaggaaaccccgggatag

SEQ ID NO: 8 - DNA, 1110 bp, Escherichia coli
atgaaattattattacttacaggtgcaacaggatttcttggtggcgcggtcctggataagctgctggataactgtaataatataaatttgctacttttagtacgagcacctactccacaagcgggactggaaagaattaaagaaaatatgcgtaaatttaatgtttgtgaggaaaggttgcatgcattaactaatgataacatcttgcctggggatctaaataatccggaagcctttctcatggatcctcgtcttgatgaagtcactcatgttataaactgtgcggctatagcttcttttggtaataatccttttatatggaatgtgaatgttacaggtacacttgcttttgcaagaagaatggcaaaagtggcaggactgaaacgcttccttcatgttggtactgctatgtcttgtacacctcatacggggtcgctagttaaggaagagtctgcttcatcagaaacaggtgaacatttagtggagtatacgcattcaaaagcaacaatagaatatctgatgcgtaagcagtgtcctgatttacctttgttggttgcccgaccatcaattattgttggccacagtcgtttagggtgcttaccttcaaccagtattttctgggtattcagaatggggttaatgttgcaaaaatttatgtgctctctggatgataaaatagatgttatccctgtagattattgtgctgatgcattgctaatgttgcttgaaagctcgttaattaatggtgagattgttcatatatcagcaggtaaagaaagtagtgtgacgttctctgctattgacgaagctgtagcccgtgctttgaactgtgatcctgttggagacagatatactaaagtcagttatgacatactggcaatgagccgtcatgattttaaaaatatttttggtccctgtaacgaacgccttatgttaaaagccattcgtttatatggagcgttcagtatgctcaatgtttgtttcagtaacgacaagctactgagtatcggaatgcctaaaccgccaaagtttactgattatattaaatactgtatagaaacgacaaaacacctttcaattcaacaacaaatggaagttgattttaaataa

SEQ ID NO: 9 - DNA, 1000 bp, Escherichia coli
agaatcacaactctcggcaatatatcatcattttgaaaatataaccccataaaaataagagtcaacataaaccaaaagtgcaccattaatcttttaatataattaactttatctaatccaattttatttataacacgtttagggttataaataaagcatgtaaagaattgagatataatgatactatacatcaaaccctcagcattgtaatgaggtattaaaaaacatgacagaattaaaaccataactgctgatataatactttgcctatgaaaatcgtaaataccaatggcagtgccaattgaggttagaataacctgacatgtttcaatatagaatataataattattgctactatataatagtaggatattacatctattttccccttaagaatatactccgcaacaggaatacctaacaatgccacaaaagaagtagaaataacagatataagcacactgatatctaatagtttaagtgtgagagggataacatcaacaccatcatggaaacgctttgagagcgtaggcatcaaataacttgcaaccaaaataattatcaaattataaacattaaatatttgcaaaaagaaaccatatataatagtagaactagaactgctttctgaaccaaatattttcaaataatatatagacaatgtatagatgaaaattgcaggaaaaacagtaaaaaaaagcttaaggttatacttgaatggtagatggaatgatttttcgctcctgttgacagacttcttatgcttaaggagtaaaaatgacaaagaatatattaagcagaatagtgagctcaaaaaccatacaagagttaaatcatacaaatcaatgtttttatcagaatgataaaacaagaaaaggaaagcagttggcataattatggcgtacagaaatcgataaactttatcgataataatattttgttttgcatatacacatgcattaataatattcgatatactacgtaccaccaaacccatac